European Patent Specification EP 3 003 339 B1, published March 22, 2023. Title: Compositions for use in cartilage degradation. Applicant: Nestec. The sequence listing filed with the application follows.

SEQUENCE LISTING (8 sequences)

SEQ ID NO: 1 - DNA, 23 bp, Bos taurus
  misc_feature: Primer
aagggcattctaggctacactga

SEQ ID NO: 2 - DNA, 24 bp, Bos taurus
  misc_feature: primer
agagtgagtgtcgctgttgaagtc

SEQ ID NO: 3 - DNA, 20 bp, Bos taurus
  misc_feature: primer
cacctcagccaccatcacag

SEQ ID NO: 4 - DNA, 20 bp, Bos taurus
  misc_feature: Primer
agtactctggcccgaaggtc

SEQ ID NO: 5 - DNA, 24 bp, Bos taurus
  misc_feature: Primer
cacccatcaatttttcaagacaga

SEQ ID NO: 6 - DNA, 20 bp, Bos taurus
  misc_feature: primer
agtactctggcccgaaggtc

SEQ ID NO: 7 - DNA, 28 bp, Bos taurus
  misc_feature: primer
gcagagagctacctgaaatcatactact

SEQ ID NO: 8 - DNA, 23 bp, Bos taurus
  misc_feature: primer
aatcacagagcttgctgcagttt